European Patent Specification EP 3 246 336 B1, published January 4, 2023. Title: Nucleic acid molecule for coding phytic Acid-Sensitive Gle1 protein mutant and use thereof. Applicant: University-Industry Foundation, Yonsei University. The sequence listing filed with the application follows.

SEQUENCE LISTING (17 sequences)

SEQ ID NO: 1 - DNA, 1836 bp, Gle 1 gene of Arabidopsis thaliana
atggggattgttttggaacctccttgtcctaaaagtgttgatgggattagcattgatcctgagcctaattggaatttcgagagtttggtcgctgagattgcttctgttgaaaagaagctcaatggcttctcaatgtatcctcagccaattactaacacaaccttacggatgggaaggagaggtggaggatttgtaatgcatgtctcagaagatgagatggagagtgacgaaggtgaagagagtgatgatgaggaagaagaagaagatcatagtcaaatctgtacagcgggaaaacgttttgcctgtgatgagctttacttgagtgatgaatctgatgaagagtttgatcatgaacctgagtatatgatgaataagttgggtctggctgagagtgccctatatgaggttatcaacgaccaccaaaccgaaatcaaggacgacattaggaatcaagtatcagttgttgaaacagaaataatgaatgagattgaaacgtctctctctgccatagcccgggttgaaaagtacagtgagactcggaaagaagttgaacggaaacttgatcttcaatatcagcgaaaagttgctgaagcacttgatacccatctgactgcagtccaacgcgaacataaaattaaatcgcaaatagaagaaagaaagataaggagcgaggaagctcaggaggaggccaggaggaaggaaagggctcatcaagaagagaaaatacgtcaagaaaaagctcgcgcagaggctcaaatgctagcaaaaatcagagctgaagaagaaaagaaagaagttgagagaaaggcagccagagaagtagctgaaaaagaagtagcagatcgcaaagctgccgaacaaaaacttgcggaacagaaggctgtgatagagagtgttacggggagttcagctacatcaaatgctcaagctgggggtaattcaatccgagctgcagaaagtgctttgatattggagaaccacagattgaaaaagctcgaagaactagaaacaacgaaccaatcgcttaagtcacgttcaaatgaaaactttagcagttttgagaagcatattggaagagtgataaggcaaataagtgggacaaaggatagtgtaagtgggaaaatcaatgatattgtgaaaatatttaaagaccctcgttgtccggtatccataagtattgcagcttttgcaaagaagatggtcaccactaaggaaaaaccaaacccttttgcatgcagctatgtcattgtttacatcaactcacagtttccccaagttatggatattcttctcgcggaattccacaaagcttgcatttacactgtcccaaagcatattgtaaactcacagtcagcttgggattcagacgcatatgaacgcctagattctataatgaggctctacggtgcacttgttcagaccgatatccgcgttggcaatgctactaacgttcatgggatagaacatggatgggcttggttagcccggttccttaacaaaatcccagccaacagagccactgcgacagccttgaactcctttctccagacggctgggtttggtcttcatcagaggtacaaatctcagtttctgaaggttgtgaatgttgtgagagagcatttcttgcagaaattgcgggcgaagaaggacacgtcggatctacttgtgatcatagccgaaatcacagcgtacttagatgaccggatgtatctcaaggaacctgaaggaagagctatgaagacgactagtaccttgtcctctgaacttactgctgaattaaatcagccgaactacaatcagaattaccagaggaatgattacagaaactactattga

SEQ ID NO: 2 - protein, 611 aa, Gle1 protein of Arabidopsis thaliana
MGIVLEPPCPKSVDGISIDPEPNWNFESLVAEIASVEKKLNGFSMYPQPITNTTLRMGRRGGGFVMHVSEDEMESDEGEESDDEEEEEDHSQICTAGKRFACDELYLSDESDEEFDHEPEYMMNKLGLAESALYEVINDHQTEIKDDIRNQVSVVETEIMNEIETSLSAIARVEKYSETRKEVERKLDLQYQRKVAEALDTHLTAVQREHKIKSQIEERKIRSEEAQEEARRKERAHQEEKIRQEKARAEAQMLAKIRAEEEKKEVERKAAREVAEKEVADRKAAEQKLAEQKAVIESVTGSSATSNAQAGGNSIRAAESALILENHRLKKLEELETTNQSLKSRSNENFSSFEKHIGRVIRQISGTKDSVSGKINDIVKIFKDPRCPVSISIAAFAKKMVTTKEKPNPFACSYVIVYINSQFPQVMDILLAEFHKACIYTVPKHIVNSQSAWDSDAYERLDSIMRLYGALVQTDIRVGNATNVHGIEHGWAWLARFLNKIPANRATATALNSFLQTAGFGLHQRYKSQFLKVVNVVREHFLQKLRAKKDTSDLLVIIAEITAYLDDRMYLKEPEGRAMKTTSTLSSELTAELNQPNYNQNYQRNDYRNYY

SEQ ID NO: 3 - DNA, 19 bp, Artificial Sequence
  Forward primer for amplifying of 356 bp Gle1 cDNA fragment
atggggattgttttggaac

SEQ ID NO: 4 - DNA, 22 bp, Artificial Sequence
  Reverse primer for amplifying of 356 bp Gle1 cDNA fragment
ggttcatgatcaaactcttcat

SEQ ID NO: 5 - DNA, 21 bp, Artificial Sequence
  Forward primer for amplifying of 330 bp Gle1 cDNA fragment
cacaaagcttgcatttacact

SEQ ID NO: 6 - DNA, 21 bp, Artificial Sequence
  Reverse primer for amplifying of 330 bp Gle1 cDNA fragment
atgctctctcacaacattcac

SEQ ID NO: 7 - DNA, 20 bp, Artificial Sequence
  Forward primer for detecting of Gle1 transcript in RNAi-Gle1(N)
catggatgggcttggttagc

SEQ ID NO: 8 - DNA, 19 bp, Artificial Sequence
  Reverse primer for detecting of Gle1 transcript in RNAi-Gle1(N)
tgtcgcagtggctctgttg

SEQ ID NO: 9 - DNA, 24 bp, Artificial Sequence
  Forward primer for detecting of Gle1 transcript in RNAi-Gle1(C)
tcagccaattactaacacaacctt

SEQ ID NO: 10 - DNA, 22 bp, Artificial Sequence
  Reverse primer for detecting of Gle1 transcript in RNAi-Gle1(C)
gacatgcattacaaatcctcca

SEQ ID NO: 11 - DNA, 21 bp, Artificial Sequence
  Forward primer for detecting of UBC10 transcript
atgggtccttcagagagtcct

SEQ ID NO: 12 - DNA, 21 bp, Artificial Sequence
  Reverse primer for detecting of UBC10 transcript
tggaacaccttggtcctaaag

SEQ ID NO: 13 - protein, 14 aa, Gle1-InsP6 binding site of Glycine max
LLAELHRACIYTVP

SEQ ID NO: 14 - protein, 14 aa, Gle1-InsP6 binding site of Oryza sativa
LLAEFHRVCMYTVP

SEQ ID NO: 15 - protein, 14 aa, Gle1-InsP6 binding site of Zea mays
LLAEFNRVCIYTVP

SEQ ID NO: 16 - protein, 14 aa, Gle1-InsP6 binding site of Hordeum vulgare
LLAEFNKVCMYTVP

SEQ ID NO: 17 - protein, 14 aa, Gle1-InsP6 binding site of Triticum aestivum
LLAEFNKVCMYTVP